European Patent Application EP 4 656 718 A2, published December 3, 2025. Title: Methods for reducing or shutting down lactation in non-human mammals and reagents therefor. Applicant: MammBio Pty Ltd. The sequence listing filed with the application follows.

SEQUENCE LISTING (3 sequences)

SEQ ID NO: 1 - DNA, 18 bp, synthetic construct
  source 1..18: mol_type = other DNA
gctcttcctaaagcagat

SEQ ID NO: 2 - DNA, 18 bp, synthetic construct
  source 1..18: mol_type = other DNA
gctcttcctaaagcagaa

SEQ ID NO: 3 - DNA, 24 bp, synthetic construct
  source 1..24: mol_type = other DNA
ggtgtcagaattcaagaagcagac